European Patent Application EP 4 248 987 A1, published September 27, 2023. Title: CHIMERIC BACTERIOCINS AND METHOD FOR THE CONTROL OF PSEUDOMONAS. Applicant: Nomad Biioscience GmbH UAB Nomads. The sequence listing filed with the application follows.

SEQUENCE LISTING (39 sequences)

SEQ ID NO: 1 - protein, 309 aa, Artificial Sequence
  Pyocin S5 first fragment
MSNDNEVPGSMVIVAQGPDDQYAYEVPPIDSAAVAGNMFGDLIQREIYLQKNIYYPVRSIFEQGTKEKKEINKKVSDQVDGLLKQITQGKREATRQERVDVMSAVLHKMESDLEGYKKTFTKGPFIDYEKQSSLSIYEAWVKIWEKNSWEERKKYPFQQLVRDELERAVAYYKQDSLSEAVKVLRQELNKQKALKEKEDLSQLERDYRTRKANLEMKVQSELDQAGSALPPLVSPTPEQWLERATRLVTQAIADKKQLQTTNNTLIKNSPTPLEKQKAIYNGELLVDEIASLQARLVKLNAETTRRRTE

SEQ ID NO: 2 - DNA, 927 bp, Artificial Sequence
  Pyocin S5 first segment coding sequence
atgtccaatgataacgaagtgccaggttcaatggttatagttgctcaaggtccagatgatcaatacgcttacgaagttcctccaatcgattctgctgctgttgctggaaatatgttcggagatcttatccaaagggaaatatatcttcaaaagaatatctattacccagttagatctatcttcgagcaaggaacaaaggaaaagaaagagattaataagaaagtttcagatcaagttgatggacttttgaagcaaattacacaaggaaagagagaagctactaggcaagagagagttgatgttatgtcagctgttcttcataagatggaatctgatttggagggatataagaaaacttttacaaagggtccttttattgattacgaaaagcaatcttcactttcaatctatgaagcttgggttaagatttgggagaaaaattcttgggaggagagaaagaaatacccttttcaacaacttgttagggatgaattggagagagctgttgcttattacaagcaagattctctttcagaagctgttaaagttcttaggcaagagttgaataagcaaaaggctttgaaggaaaaggaggatctttcacaattggaaagagattacaggacaagaaaggctaatcttgagatgaaggttcaatctgagttggatcaagctggatcagctcttccacctttggtttctccaactcctgaacaatggcttgagagggctacaagattggttactcaagctattgctgataagaaacaacttcaaactacaaataacacattgattaagaactctccaactcctcttgaaaagcaaaaagctatctataatggtgaacttttggttgatgagattgcttcattgcaagctaggcttgttaaattgaatgctgagactacaagaaggagaacagaa

SEQ ID NO: 3 - protein, 192 aa, Artificial Sequence
  PmnH second segment
KELTPDEKAAYTDAVSFVSTANEQMLQKYGANLSKVAQDMQAEIAGKKVRSYAEAMATFEKISANPAMKLNALDTQAVVDALNALDKASFADNITRLGKAFGVVGKVVQAEAIREKTVSGFQTGDWKPLMLELEAMAVGTGAGILLATSMAFFFPVFASAAAGVVVVALMMAATAAYFDAAKVDEINNLILN

SEQ ID NO: 4 - DNA, 579 bp, Artificial Sequence
  PmnH second segment coding sequence
aaggaacttacaccagatgagaaagctgcttatactgatgctgtttcttttgtttcaacagctaatgagcaaatgttgcaaaagtacggtgctaatctttcaaaagttgctcaagatatgcaagctgagattgctggaaagaaagttaggtcttatgctgaagctatggctacttttgagaagatttcagctaatccagctatgaaacttaatgctttggatacacaagctgttgttgatgctcttaatgctttggataaggcttctttcgctgataacatcactaggttgggaaaggcttttggtgttgttggaaaagttgttcaagctgaagctattagagagaagacagtttcaggttttcaaactggagattggaaacctttgatgcttgaattggaggctatggctgttggaactggtgctggaattcttttggctacatctatggctttctttttcccagtttttgcttcagctgctgctggagttgttgttgttgctcttatgatggctgctacagctgcttactttgatgctgctaaggttgatgaaattaataaccttattttgaattaa

SEQ ID NO: 5 - protein, 501 aa, Artificial Sequence
  Chimeric S5-PmnH
MSNDNEVPGSMVIVAQGPDDQYAYEVPPIDSAAVAGNMFGDLIQREIYLQKNIYYPVRSIFEQGTKEKKEINKKVSDQVDGLLKQITQGKREATRQERVDVMSAVLHKMESDLEGYKKTFTKGPFIDYEKQSSLSIYEAWVKIWEKNSWEERKKYPFQQLVRDELERAVAYYKQDSLSEAVKVLRQELNKQKALKEKEDLSQLERDYRTRKANLEMKVQSELDQAGSALPPLVSPTPEQWLERATRLVTQAIADKKQLQTTNNTLIKNSPTPLEKQKAIYNGELLVDEIASLQARLVKLNAETTRRRTEKELTPDEKAAYTDAVSFVSTANEQMLQKYGANLSKVAQDMQAEIAGKKVRSYAEAMATFEKISANPAMKLNALDTQAVVDALNALDKASFADNITRLGKAFGVVGKVVQAEAIREKTVSGFQTGDWKPLMLELEAMAVGTGAGILLATSMAFFFPVFASAAAGVVVVALMMAATAAYFDAAKVDEINNLILN

SEQ ID NO: 6 - DNA, 1506 bp, Artificial Sequence
  S5-PmnH coding sequence
atgtccaatgataacgaagtgccaggttcaatggttatagttgctcaaggtccagatgatcaatacgcttacgaagttcctccaatcgattctgctgctgttgctggaaatatgttcggagatcttatccaaagggaaatatatcttcaaaagaatatctattacccagttagatctatcttcgagcaaggaacaaaggaaaagaaagagattaataagaaagtttcagatcaagttgatggacttttgaagcaaattacacaaggaaagagagaagctactaggcaagagagagttgatgttatgtcagctgttcttcataagatggaatctgatttggagggatataagaaaacttttacaaagggtccttttattgattacgaaaagcaatcttcactttcaatctatgaagcttgggttaagatttgggagaaaaattcttgggaggagagaaagaaatacccttttcaacaacttgttagggatgaattggagagagctgttgcttattacaagcaagattctctttcagaagctgttaaagttcttaggcaagagttgaataagcaaaaggctttgaaggaaaaggaggatctttcacaattggaaagagattacaggacaagaaaggctaatcttgagatgaaggttcaatctgagttggatcaagctggatcagctcttccacctttggtttctccaactcctgaacaatggcttgagagggctacaagattggttactcaagctattgctgataagaaacaacttcaaactacaaataacacattgattaagaactctccaactcctcttgaaaagcaaaaagctatctataatggtgaacttttggttgatgagattgcttcattgcaagctaggcttgttaaattgaatgctgagactacaagaaggagaacagaaaaggaacttacaccagatgagaaagctgcttatactgatgctgtttcttttgtttcaacagctaatgagcaaatgttgcaaaagtacggtgctaatctttcaaaagttgctcaagatatgcaagctgagattgctggaaagaaagttaggtcttatgctgaagctatggctacttttgagaagatttcagctaatccagctatgaaacttaatgctttggatacacaagctgttgttgatgctcttaatgctttggataaggcttctttcgctgataacatcactaggttgggaaaggcttttggtgttgttggaaaagttgttcaagctgaagctattagagagaagacagtttcaggttttcaaactggagattggaaacctttgatgcttgaattggaggctatggctgttggaactggtgctggaattcttttggctacatctatggctttctttttcccagtttttgcttcagctgctgctggagttgttgttgttgctcttatgatggctgctacagctgcttactttgatgctgctaaggttgatgaaattaataaccttattttgaattaa

SEQ ID NO: 7 - protein, 189 aa, Artificial Sequence
  Pflu095 second segment
KDKVRTEVVDIEAAIKFTSDFYAEAGVRFGDSASKLASDLADSAQGKKIRSADEAFKAFDKYKNELDKKFSVKDRAAAAKYIDSIDYEAIGKAATKFSKGLGYVGPVIDAKDSIIEFINSMESGDWKPFFLKLESIALGLAATAFVGIAFGFIATTPMGILAFAFIVAATGAAIDDNFAEKLNKFVSSL

SEQ ID NO: 8 - DNA, 570 bp, Artificial Sequence
  Pflu095 second segment coding sequence
aaggataaggttaggactgaggtggtggacatcgaggctgctattaagttcaccagcgacttctatgctgaggctggtgttaggttcggcgactctgcttctaagcttgctagcgatcttgctgatagcgcccagggtaagaaaatcaggtctgctgatgaggctttcaaggccttcgacaagtacaagaacgagctggacaagaagttcagcgtcaaggatagagctgctgccgctaagtacatcgacagcattgattacgaggctatcggcaaggctgccaccaagttctctaaaggtcttggttacgtgggccctgtgatcgatgctaaggatagcatcatcgagttcatcaacagcatggaaagcggcgactggaagccattcttcctgaagcttgagtctatcgctctgggtcttgctgctactgctttcgtgggtattgccttcggtttcattgctactacccctatgggtatcctggccttcgcttttattgtggctgctaccggtgctgctatcgacgataatttcgctgagaagctgaacaagttcgtgtccagcctttaa

SEQ ID NO: 9 - protein, 498 aa, Artificial Sequence
  S5-Pflu095
MSNDNEVPGSMVIVAQGPDDQYAYEVPPIDSAAVAGNMFGDLIQREIYLQKNIYYPVRSIFEQGTKEKKEINKKVSDQVDGLLKQITQGKREATRQERVDVMSAVLHKMESDLEGYKKTFTKGPFIDYEKQSSLSIYEAWVKIWEKNSWEERKKYPFQQLVRDELERAVAYYKQDSLSEAVKVLRQELNKQKALKEKEDLSQLERDYRTRKANLEMKVQSELDQAGSALPPLVSPTPEQWLERATRLVTQAIADKKQLQTTNNTLIKNSPTPLEKQKAIYNGELLVDEIASLQARLVKLNAETTRRRTEKDKVRTEVVDIEAAIKFTSDFYAEAGVRFGDSASKLASDLADSAQGKKIRSADEAFKAFDKYKNELDKKFSVKDRAAAAKYIDSIDYEAIGKAATKFSKGLGYVGPVIDAKDSIIEFINSMESGDWKPFFLKLESIALGLAATAFVGIAFGFIATTPMGILAFAFIVAATGAAIDDNFAEKLNKFVSSL

SEQ ID NO: 10 - DNA, 1497 bp, Artificial Sequence
  S5-Pflu095 coding sequence
atgtccaatgataacgaagtgccaggttcaatggttatagttgctcaaggtccagatgatcaatacgcttacgaagttcctccaatcgattctgctgctgttgctggaaatatgttcggagatcttatccaaagggaaatatatcttcaaaagaatatctattacccagttagatctatcttcgagcaaggaacaaaggaaaagaaagagattaataagaaagtttcagatcaagttgatggacttttgaagcaaattacacaaggaaagagagaagctactaggcaagagagagttgatgttatgtcagctgttcttcataagatggaatctgatttggagggatataagaaaacttttacaaagggtccttttattgattacgaaaagcaatcttcactttcaatctatgaagcttgggttaagatttgggagaaaaattcttgggaggagagaaagaaatacccttttcaacaacttgttagggatgaattggagagagctgttgcttattacaagcaagattctctttcagaagctgttaaagttcttaggcaagagttgaataagcaaaaggctttgaaggaaaaggaggatctttcacaattggaaagagattacaggacaagaaaggctaatcttgagatgaaggttcaatctgagttggatcaagctggatcagctcttccacctttggtttctccaactcctgaacaatggcttgagagggctacaagattggttactcaagctattgctgataagaaacaacttcaaactacaaataacacattgattaagaactctccaactcctcttgaaaagcaaaaagctatctataatggtgaacttttggttgatgagattgcttcattgcaagctaggcttgttaaattgaatgctgagactacaagaaggagaacagaaaaggataaggttaggactgaggtggtggacatcgaggctgctattaagttcaccagcgacttctatgctgaggctggtgttaggttcggcgactctgcttctaagcttgctagcgatcttgctgatagcgcccagggtaagaaaatcaggtctgctgatgaggctttcaaggccttcgacaagtacaagaacgagctggacaagaagttcagcgtcaaggatagagctgctgccgctaagtacatcgacagcattgattacgaggctatcggcaaggctgccaccaagttctctaaaggtcttggttacgtgggccctgtgatcgatgctaaggatagcatcatcgagttcatcaacagcatggaaagcggcgactggaagccattcttcctgaagcttgagtctatcgctctgggtcttgctgctactgctttcgtgggtattgccttcggtttcattgctactacccctatgggtatcctggccttcgcttttattgtggctgctaccggtgctgctatcgacgataatttcgctgagaagctgaacaagttcgtgtccagcctttaa

SEQ ID NO: 11 - protein, 191 aa, Artificial Sequence
  Pflu373 second segment
AEEQAKAEEEIKGAIKFTADFYKEIGEKYGAQMTASATDLAETAKGKTLRSAEEALKAFDQYKDHLDKKFSAADRAAIVNALDSLDRAELAKNLNLFAKGFGYTSKAFDVYDLVEEVKKSYASGDWNNTALKVETLFAGSAATGLIAFAFGVTVSTPVGIVAFALIMALVSAYIDDAHVKQFNDALDAILP

SEQ ID NO: 12 - DNA, 576 bp, Artificial Sequence
  Pflu373 second segment coding sequence
gctgaggaacaggctaaggctgaggaagagattaagggcgctatcaagttcaccgccgacttctacaaagaaatcggcgagaagtacggcgctcagatgactgcttctgctactgatcttgctgagactgctaagggtaagacccttaggtcagcagaagaggctctgaaggctttcgatcagtacaaggatcacctggacaagaagttcagcgctgctgatagggctgctattgtgaacgctctggattctcttgacagggctgagcttgctaagaacctgaacctgttcgctaaaggcttcggctacacctctaaggcattcgatgtgtacgatctggtggaagaggtgaagaaaagctacgctagcggcgattggaacaacaccgctcttaaggttgagactctgttcgctggttctgctgctaccggtttgattgctttcgctttcggtgtgactgtgtctacccctgttggtattgtggctttcgctctgattatggctctggtgagcgcttacatcgatgacgctcatgtgaagcagttcaacgatgctctggatgctatcctgccttaa

SEQ ID NO: 13 - protein, 500 aa, Artificial Sequence
  S5-Pflu373
MSNDNEVPGSMVIVAQGPDDQYAYEVPPIDSAAVAGNMFGDLIQREIYLQKNIYYPVRSIFEQGTKEKKEINKKVSDQVDGLLKQITQGKREATRQERVDVMSAVLHKMESDLEGYKKTFTKGPFIDYEKQSSLSIYEAWVKIWEKNSWEERKKYPFQQLVRDELERAVAYYKQDSLSEAVKVLRQELNKQKALKEKEDLSQLERDYRTRKANLEMKVQSELDQAGSALPPLVSPTPEQWLERATRLVTQAIADKKQLQTTNNTLIKNSPTPLEKQKAIYNGELLVDEIASLQARLVKLNAETTRRRTEAEEQAKAEEEIKGAIKFTADFYKEIGEKYGAQMTASATDLAETAKGKTLRSAEEALKAFDQYKDHLDKKFSAADRAAIVNALDSLDRAELAKNLNLFAKGFGYTSKAFDVYDLVEEVKKSYASGDWNNTALKVETLFAGSAATGLIAFAFGVTVSTPVGIVAFALIMALVSAYIDDAHVKQFNDALDAILP

SEQ ID NO: 14 - DNA, 2791 bp, Artificial Sequence
  S5-Pflu373 coding sequence
atgtccaatgataacgaagtgccaggttcaatggttatagttgctcaaggtccagatgatcaatacgcttacgaagttcctccaatcgattctgctgctgttgctggaaatatgttcggagatcttatccaaagggaaatatatcttcaaaagaatatctattacccagttagatctatcttcgagcaaggaacaaaggaaaagaaagagattaataagaaagtttcagatcaagttgatggacttttgaagcaaattacacaaggaaagagagaagctactaggcaagagagagttgatgttatgtcagctgttcttcataagatggaatctgatttggagggatataagaaaacttttacaaagggtccttttattgattacgaaaagcaatcttcactttcaatctatgaagcttgggttaagatttgggagaaaaattcttgggaggagagaaagaaatacccttttcaacaacttgttagggatgaattggagagagctgttgcttattacaagcaagattctctttcagaagctgttaaagttcttaggcaagagttgaataagcaaaaggctttgaaggaaaaggaggatctttcacaattggaaagagattacaggacaagaaaggctaatcttgagatgaaggttcaatctgagttggatcaagctggatcagctcttccacctttggtttctccaactcctgaacaatggcttgagagggctacaagattggttactcaagctattgctgataagaaacaacttcaaactacaaataacacattgattaagaactctccaactcctcttgaaaagcaaaaagctatctataatggtgaacttttggttgatgagattgcttcattgcaagctaggcttgttaaattgaatgctgagactacaagaaggagaacagaagctgaggaacaggctaaggctgaggaagagattaagggcgctatcaagttcaccgccgacttctacaaagaaatcggcgagaagtacggcgctcagatgactgcttctgctactgatcttgctgagactgctaagggtaagacccttaggtcagcagaagaggctctgaaggctttcgatcagtacaaggatcacctggacaagaagttcagcgctgctgatagggctgctattgtgaacgctctggattctcttgacagggctgagcttgctaagaacctgaacctgttcgctaaaggcttcggctacacctctaaggcattcgatgtgtacgatctggtggaagaggtgaagaaaagctatgtccaatgataacgaagtgccaggttcaatggttatagttgctcaaggtccagatgatcaatacgcttacgaagttcctccaatcgattctgctgctgttgctggaaatatgttcggagatcttatccaaagggaaatatatcttcaaaagaatatctattacccagttagatctatcttcgagcaaggaacaaaggaaaagaaagagattaataagaaagtttcagatcaagttgatggacttttgaagcaaattacacaaggaaagagagaagctactaggcaagagagagttgatgttatgtcagctgttcttcataagatggaatctgatttggagggatataagaaaacttttacaaagggtccttttattgattacgaaaagcaatcttcactttcaatctatgaagcttgggttaagatttgggagaaaaattcttgggaggagagaaagaaatacccttttcaacaacttgttagggatgaattggagagagctgttgcttattacaagcaagattctctttcagaagctgttaaagttcttaggcaagagttgaataagcaaaaggctttgaaggaaaaggaggatctttcacaattggaaagagattacaggacaagaaaggctaatcttgagatgaaggttcaatctgagttggatcaagctggatcagctcttccacctttggtttctccaactcctgaacaatggcttgagagggctacaagattggttactcaagctattgctgataagaaacaacttcaaactacaaataacacattgattaagaactctccaactcctcttgaaaagcaaaaagctatctataatggtgaacttttggttgatgagattgcttcattgcaagctaggcttgttaaattgaatgctgagactacaagaaggagaacagaagctgaggaacaggctaaggctgaggaagagattaagggcgctatcaagttcaccgccgacttctacaaagaaatcggcgagaagtacggcgctcagatgactgcttctgctactgatcttgctgagactgctaagggtaagacccttaggtcagcagaagaggctctgaaggctttcgatcagtacaaggatcacctggacaagaagttcagcgctgctgatagggctgctattgtgaacgctctggattctcttgacagggctgagcttgctaagaacctgaacctgttcgctaaaggcttcggctacacctctaaggcattcgatgtgtacgatctggtggaagaggtgaagaaaagctacgctagcggcgattggaacaacaccgctcttaaggttgagactctgttcgctggttctgctgctaccggtttgattgctttcgctttcggtgtgactgtgtctacccctgttggtattgtggctttcgctctgattatggctctggtgagcgcttacatcgatgacgctcatgtgaagcagttcaacgatgctctggatgctatcctgccttaa

SEQ ID NO: 15 - protein, 189 aa, Artificial Sequence
  Pflu794 second segment
KASDQANNVDIEEAILFTTTFYENLTEKYGEKVSAVAKELAESAKGKTMRSSKEALQTFEKYKDTYNGRFRSRDRREVDRALKSLDKELLSKNLAKFSKAFGSVSKIGDLTEVFIELENSIRTGDWKPLLLTLEGIGLGMAGTYLVAAVFGISATTPLGIVVFAVLMAATSAYIDDDLVKKVNKDLFGF

SEQ ID NO: 16 - DNA, 570 bp, Artificial Sequence
  Pflu794 second segment coding sequence
aaggctagcgaccaggctaacaacgttgacatcgaagaggctatcctgttcaccaccaccttctacgagaacctcactgagaagtacggcgagaaggttagcgctgtggctaaagaacttgctgagagcgctaagggcaagaccatgaggtcatctaaagaggctctgcagaccttcgagaagtacaaggatacctacaacggccggttcaggtctagggatagaagggaagttgatcgggctctgaagtcccttgacaaagagctgctgtctaagaacctcgccaagttctctaaggctttcggctccgtgtctaagatcggtgatcttaccgaggtgttcatcgagttggagaactctatcaggaccggcgattggaagcctcttctgcttacccttgaaggtatcggtcttggtatggctggaacctaccttgttgctgctgtgttcggtatctctgctactacccctcttggcattgtggtgttcgctgttcttatggctgctaccagcgcttacatcgatgatgacctggtgaagaaggtgaacaaggacctgttcggcttctaa

SEQ ID NO: 17 - protein, 498 aa, Artificial Sequence
  S5-Pflu794
MSNDNEVPGSMVIVAQGPDDQYAYEVPPIDSAAVAGNMFGDLIQREIYLQKNIYYPVRSIFEQGTKEKKEINKKVSDQVDGLLKQITQGKREATRQERVDVMSAVLHKMESDLEGYKKTFTKGPFIDYEKQSSLSIYEAWVKIWEKNSWEERKKYPFQQLVRDELERAVAYYKQDSLSEAVKVLRQELNKQKALKEKEDLSQLERDYRTRKANLEMKVQSELDQAGSALPPLVSPTPEQWLERATRLVTQAIADKKQLQTTNNTLIKNSPTPLEKQKAIYNGELLVDEIASLQARLVKLNAETTRRRTEKASDQANNVDIEEAILFTTTFYENLTEKYGEKVSAVAKELAESAKGKTMRSSKEALQTFEKYKDTYNGRFRSRDRREVDRALKSLDKELLSKNLAKFSKAFGSVSKIGDLTEVFIELENSIRTGDWKPLLLTLEGIGLGMAGTYLVAAVFGISATTPLGIVVFAVLMAATSAYIDDDLVKKVNKDLFGF

SEQ ID NO: 18 - DNA, 1497 bp, Artificial Sequence
  S5-Pflu794 coding sequence
atgtccaatgataacgaagtgccaggttcaatggttatagttgctcaaggtccagatgatcaatacgcttacgaagttcctccaatcgattctgctgctgttgctggaaatatgttcggagatcttatccaaagggaaatatatcttcaaaagaatatctattacccagttagatctatcttcgagcaaggaacaaaggaaaagaaagagattaataagaaagtttcagatcaagttgatggacttttgaagcaaattacacaaggaaagagagaagctactaggcaagagagagttgatgttatgtcagctgttcttcataagatggaatctgatttggagggatataagaaaacttttacaaagggtccttttattgattacgaaaagcaatcttcactttcaatctatgaagcttgggttaagatttgggagaaaaattcttgggaggagagaaagaaatacccttttcaacaacttgttagggatgaattggagagagctgttgcttattacaagcaagattctctttcagaagctgttaaagttcttaggcaagagttgaataagcaaaaggctttgaaggaaaaggaggatctttcacaattggaaagagattacaggacaagaaaggctaatcttgagatgaaggttcaatctgagttggatcaagctggatcagctcttccacctttggtttctccaactcctgaacaatggcttgagagggctacaagattggttactcaagctattgctgataagaaacaacttcaaactacaaataacacattgattaagaactctccaactcctcttgaaaagcaaaaagctatctataatggtgaacttttggttgatgagattgcttcattgcaagctaggcttgttaaattgaatgctgagactacaagaaggagaacagaaaaggctagcgaccaggctaacaacgttgacatcgaagaggctatcctgttcaccaccaccttctacgagaacctcactgagaagtacggcgagaaggttagcgctgtggctaaagaacttgctgagagcgctaagggcaagaccatgaggtcatctaaagaggctctgcagaccttcgagaagtacaaggatacctacaacggccggttcaggtctagggatagaagggaagttgatcgggctctgaagtcccttgacaaagagctgctgtctaagaacctcgccaagttctctaaggctttcggctccgtgtctaagatcggtgatcttaccgaggtgttcatcgagttggagaactctatcaggaccggcgattggaagcctcttctgcttacccttgaaggtatcggtcttggtatggctggaacctaccttgttgctgctgtgttcggtatctctgctactacccctcttggcattgtggtgttcgctgttcttatggctgctaccagcgcttacatcgatgatgacctggtgaagaaggtgaacaaggacctgttcggcttctaa

SEQ ID NO: 19 - protein, 202 aa, Artificial Sequence
  Pflu618 second segment
AEAEAKRIDDYKRAVAFVADANKYILEKYGANLHQVVMDLQKDISGKKIRSYAEAMQTFEAVRTNPNARLSPQDTRAVVDALNALDKATYMDSVNKLAKGFGVTGKIVQAHSVIEKTVIGFRDGNWKPLILELESIALGAGAGAAVATLLAVFSPGFAASAIGIVAVGVAIATIASLLNADNVEKINVFISDHLETALKEQR

SEQ ID NO: 20 - DNA, 609 bp, Artificial Sequence
  Pflu618 second segment coding sequence
gctgaagctgaggctaagagaattgatgattacaaaagggctgttgctttcgttgctgatgctaataagtacatcttggaaaagtacggtgctaatcttcatcaagttgttatggatttgcaaaaggatatctctggaaagaaaattagatcatacgctgaagctatgcaaacttttgaggctgttagaacaaatccaaatgctaggctttctcctcaagatactagggctgttgttgatgctttgaatgctcttgataaggctacatacatggattctgttaataagttggctaaaggatttggtgttactggaaagattgttcaagctcattcagttattgaaaagacagttattggttttagagatggaaattggaaaccacttattttggaacttgagtcaattgctttgggagctggtgctggagctgctgttgctacacttttggctgttttctctcctggatttgctgcttcagctattggtattgttgctgttggagttgctattgctactattgcttctcttttgaacgctgataacgttgagaagattaatgtttttatttcagatcatttggaaacagctcttaaagagcaaaggtaa

SEQ ID NO: 21 - protein, 511 aa, Artificial Sequence
  S5-Pflu618
MSNDNEVPGSMVIVAQGPDDQYAYEVPPIDSAAVAGNMFGDLIQREIYLQKNIYYPVRSIFEQGTKEKKEINKKVSDQVDGLLKQITQGKREATRQERVDVMSAVLHKMESDLEGYKKTFTKGPFIDYEKQSSLSIYEAWVKIWEKNSWEERKKYPFQQLVRDELERAVAYYKQDSLSEAVKVLRQELNKQKALKEKEDLSQLERDYRTRKANLEMKVQSELDQAGSALPPLVSPTPEQWLERATRLVTQAIADKKQLQTTNNTLIKNSPTPLEKQKAIYNGELLVDEIASLQARLVKLNAETTRRRTEAEAEAKRIDDYKRAVAFVADANKYILEKYGANLHQVVMDLQKDISGKKIRSYAEAMQTFEAVRTNPNARLSPQDTRAVVDALNALDKATYMDSVNKLAKGFGVTGKIVQAHSVIEKTVIGFRDGNWKPLILELESIALGAGAGAAVATLLAVFSPGFAASAIGIVAVGVAIATIASLLNADNVEKINVFISDHLETALKEQR

SEQ ID NO: 22 - DNA, 1536 bp, Artificial Sequence
  S5-Pflu618 coding sequence
atgtccaatgataacgaagtgccaggttcaatggttatagttgctcaaggtccagatgatcaatacgcttacgaagttcctccaatcgattctgctgctgttgctggaaatatgttcggagatcttatccaaagggaaatatatcttcaaaagaatatctattacccagttagatctatcttcgagcaaggaacaaaggaaaagaaagagattaataagaaagtttcagatcaagttgatggacttttgaagcaaattacacaaggaaagagagaagctactaggcaagagagagttgatgttatgtcagctgttcttcataagatggaatctgatttggagggatataagaaaacttttacaaagggtccttttattgattacgaaaagcaatcttcactttcaatctatgaagcttgggttaagatttgggagaaaaattcttgggaggagagaaagaaatacccttttcaacaacttgttagggatgaattggagagagctgttgcttattacaagcaagattctctttcagaagctgttaaagttcttaggcaagagttgaataagcaaaaggctttgaaggaaaaggaggatctttcacaattggaaagagattacaggacaagaaaggctaatcttgagatgaaggttcaatctgagttggatcaagctggatcagctcttccacctttggtttctccaactcctgaacaatggcttgagagggctacaagattggttactcaagctattgctgataagaaacaacttcaaactacaaataacacattgattaagaactctccaactcctcttgaaaagcaaaaagctatctataatggtgaacttttggttgatgagattgcttcattgcaagctaggcttgttaaattgaatgctgagactacaagaaggagaacagaagctgaagctgaggctaagagaattgatgattacaaaagggctgttgctttcgttgctgatgctaataagtacatcttggaaaagtacggtgctaatcttcatcaagttgttatggatttgcaaaaggatatctctggaaagaaaattagatcatacgctgaagctatgcaaacttttgaggctgttagaacaaatccaaatgctaggctttctcctcaagatactagggctgttgttgatgctttgaatgctcttgataaggctacatacatggattctgttaataagttggctaaaggatttggtgttactggaaagattgttcaagctcattcagttattgaaaagacagttattggttttagagatggaaattggaaaccacttattttggaacttgagtcaattgctttgggagctggtgctggagctgctgttgctacacttttggctgttttctctcctggatttgctgcttcagctattggtattgttgctgttggagttgctattgctactattgcttctcttttgaacgctgataacgttgagaagattaatgtttttatttcagatcatttggaaacagctcttaaagagcaaaggtaa

SEQ ID NO: 23 - protein, 201 aa, Artificial Sequence
  Ppu259 second segment
AEAEAKRIDDYKRAVAYVADANKFILEKYGAKLHQVVMDLQKDVSGKKIRSYNEALRTFEQVRTNPNARLSPQDTRAVVDALNALDKATYMDSVNRLAKGFGVTGKIVQAHSVVEKAIIGFQDGNWKPLLLEFESIAAGAGAGLLVALIAPPVLAAFSFPPVIAVVATGLLVAGVAALLDAKTVEKINDTIFTLVETTPAH

SEQ ID NO: 24 - DNA, 606 bp, Artificial Sequence
  Ppu259 second segment coding sequenc
gcagaggctgaggctaagaggatcgatgattacaagcgggctgttgcttacgtggccgatgctaacaagttcatcctcgagaagtacggtgccaagcttcatcaggtggtgatggatctgcagaaggacgttagcggcaagaaaatccggtcttacaacgaggctcttaggacctttgagcaggtcaggactaatcctaacgctaggttgtctcctcaggacactagggctgttgtggatgctcttaacgctctggacaaggccacctacatggattctgtgaacaggctggctaaaggtttcggtgtgaccggtaagattgtgcaggctcattctgtggtcgagaaggctattatcggtttccaggatggcaactggaagcctcttttgctcgagttcgagtctattgctgctggtgctggtgcaggtttgcttgtggctcttattgctcctcctgtgctggctgctttttctttcccacctgtgattgctgtggtggctactggtcttttggttgctggtgttgctgctctgcttgacgctaagactgtcgagaagatcaacgacaccatcttcaccctggttgagactactcctgctcactaa

SEQ ID NO: 25 - protein, 510 aa, Artificial Sequence
  S5- Ppu25
MSNDNEVPGSMVIVAQGPDDQYAYEVPPIDSAAVAGNMFGDLIQREIYLQKNIYYPVRSIFEQGTKEKKEINKKVSDQVDGLLKQITQGKREATRQERVDVMSAVLHKMESDLEGYKKTFTKGPFIDYEKQSSLSIYEAWVKIWEKNSWEERKKYPFQQLVRDELERAVAYYKQDSLSEAVKVLRQELNKQKALKEKEDLSQLERDYRTRKANLEMKVQSELDQAGSALPPLVSPTPEQWLERATRLVTQAIADKKQLQTTNNTLIKNSPTPLEKQKAIYNGELLVDEIASLQARLVKLNAETTRRRTEAEAEAKRIDDYKRAVAYVADANKFILEKYGAKLHQVVMDLQKDVSGKKIRSYNEALRTFEQVRTNPNARLSPQDTRAVVDALNALDKATYMDSVNRLAKGFGVTGKIVQAHSVVEKAIIGFQDGNWKPLLLEFESIAAGAGAGLLVALIAPPVLAAFSFPPVIAVVATGLLVAGVAALLDAKTVEKINDTIFTLVETTPAH

SEQ ID NO: 26 - DNA, 1533 bp, Artificial Sequence
  S5-Ppu259 coding sequence
atgtccaatgataacgaagtgccaggttcaatggttatagttgctcaaggtccagatgatcaatacgcttacgaagttcctccaatcgattctgctgctgttgctggaaatatgttcggagatcttatccaaagggaaatatatcttcaaaagaatatctattacccagttagatctatcttcgagcaaggaacaaaggaaaagaaagagattaataagaaagtttcagatcaagttgatggacttttgaagcaaattacacaaggaaagagagaagctactaggcaagagagagttgatgttatgtcagctgttcttcataagatggaatctgatttggagggatataagaaaacttttacaaagggtccttttattgattacgaaaagcaatcttcactttcaatctatgaagcttgggttaagatttgggagaaaaattcttgggaggagagaaagaaatacccttttcaacaacttgttagggatgaattggagagagctgttgcttattacaagcaagattctctttcagaagctgttaaagttcttaggcaagagttgaataagcaaaaggctttgaaggaaaaggaggatctttcacaattggaaagagattacaggacaagaaaggctaatcttgagatgaaggttcaatctgagttggatcaagctggatcagctcttccacctttggtttctccaactcctgaacaatggcttgagagggctacaagattggttactcaagctattgctgataagaaacaacttcaaactacaaataacacattgattaagaactctccaactcctcttgaaaagcaaaaagctatctataatggtgaacttttggttgatgagattgcttcattgcaagctaggcttgttaaattgaatgctgagactacaagaaggagaacagaagcagaggctgaggctaagaggatcgatgattacaagcgggctgttgcttacgtggccgatgctaacaagttcatcctcgagaagtacggtgccaagcttcatcaggtggtgatggatctgcagaaggacgttagcggcaagaaaatccggtcttacaacgaggctcttaggacctttgagcaggtcaggactaatcctaacgctaggttgtctcctcaggacactagggctgttgtggatgctcttaacgctctggacaaggccacctacatggattctgtgaacaggctggctaaaggtttcggtgtgaccggtaagattgtgcaggctcattctgtggtcgagaaggctattatcggtttccaggatggcaactggaagcctcttttgctcgagttcgagtctattgctgctggtgctggtgcaggtttgcttgtggctcttattgctcctcctgtgctggctgctttttctttcccacctgtgattgctgtggtggctactggtcttttggttgctggtgttgctgctctgcttgacgctaagactgtcgagaagatcaacgacaccatcttcaccctggttgagactactcctgctcactaa

SEQ ID NO: 27 - DNA, 26 bp, Artificial Sequence
  S5 fwd
aaaggtctcacatgtccaatgataac

SEQ ID NO: 28 - DNA, 33 bp, Artificial Sequence
  S5 rev
aaaggtctcattctgttctccttcttgtagtct

SEQ ID NO: 29 - DNA, 37 bp, Artificial Sequence
  PmnH fwd
aaaggtctcaagaaaaggaacttacaccagatgagaa

SEQ ID NO: 30 - DNA, 29 bp, Artificial Sequence
  PmnH rev
aaaggtctcaaagcttaattcaaaataag

SEQ ID NO: 31 - DNA, 36 bp, Artificial Sequence
  Pflu095 fwd
aaaggtctcaagaaaaggataaggttaggactgagg

SEQ ID NO: 32 - DNA, 25 bp, Artificial Sequence
  Pflu095 rev
aaaggtctcaaagcttaaaggctgg

SEQ ID NO: 33 - DNA, 35 bp, Artificial Sequence
  Pflu794 fwd
aaaggtctcaagaaaaggctagcgaccaggctaac

SEQ ID NO: 34 - DNA, 25 bp, Artificial Sequence
  Pflu794 rev
aaaggtctcaaagcttagaagccga

SEQ ID NO: 35 - DNA, 35 bp, Artificial Sequence
  Pflu618 fwd
aaaggtctcaagaagctgaagctgaggctaagaga

SEQ ID NO: 36 - DNA, 26 bp, Artificial Sequence
  Pflu618 rev
aaaggtctcaaagcttacctttgctc

SEQ ID NO: 37 - DNA, 34 bp, Artificial Sequence
  Pput259 fwd
aaaggtctcaagaagcagaggctgaggctaagag

SEQ ID NO: 38 - DNA, 25 bp, Artificial Sequence
  Pput259 rev
aaaggtctcaaagcttagtgagcag

SEQ ID NO: 39 - protein, 189 aa, Pseudomonas aeruginosa
AERKAAEEQALQDAIKFTADFYKEVTEKFGARTSEMARQLAEGARGKNIRSSAEAIKSFEKHKDALNKKLSLKDRQAIAKAFDSLDKQMMAKSLEKFSKGFGVVGKAIDAASLYQEFKISTETGDWKPFFVKIETLAAGAAASWLVGIAFATATATPIGILGFALVMAVTGAMIDEDLLEKANNLVISI